European Patent Application EP 4 230 791 A1, published August 23, 2023. Title: A bleaching process. Applicant: AB Enzymes GmbH. The sequence listing filed with the application follows.

SEQUENCE LISTING (3 sequences)

SEQ ID NO: 1 - protein, 220 aa, Artificial Sequence
  variant
DTTITQNQTGYDNGYFYSFWTDAPGTVSMTLHSGGSYSTSWRNTGNFVAGKGWSTGGRRTVTYNASFNPSGNAYLTLYGWTRNPLVEYYIVESWGTYRPTGTYKGTVTTDGGTYDIYETWRYNAPSIEGTRTFQQFWSVRQQKRTSGTITIGNHFDAWARAGMNLGSHDYQIMATEGYQSSGSSTVSISEGGNPGNPGNPGNPGNPGNPGNPGGGCVATL

SEQ ID NO: 2 - protein, 220 aa, Artificial Sequence
  variant
DTCITQNQTGYDNGYFYSFWTDSPGTVIMCLHSGGSYSTSWRNTGNFVAGKGWSTGGRRTVTYNASFNPSGNAYLTLYGWTRNPLVEYYIVESWGTYRPTGTYKGTVTTDGGTYDIYETWRYNAPSIEGTRTFQQFWSVRQQKRTSGTITIGNHFDAWARAGMNLGSHDYQIMATEGYQSSGSSTVSISEGGNPGNPGNPGNPGNPGNPGNPGGGCVATL

SEQ ID NO: 3 - protein, 301 aa, Thermopolyspora flexuosa
DTTITQNQTGYDNGYFYSFWTDAPGTVSMTLHSGGSYSTSWRNTGNFVAGKGWSTGGRRTVTYNASFNPSGNAYLTLYGWTRNPLVEYYIVESWGTYRPTGTYKGTVTTDGGTYDIYETWRYNAPSIEGTRTFQQFWSVRQQKRTSGTITIGNHFDAWARAGMNLGSHDYQIMATEGYQSSGSSTVSISEGGNPGNPGNPGNPGNPGNPGNPGGGCVATLSAGQQWSDRYNLNVSVSGSNNWTVRMDVPYPARIIATWNIHAQWPESQVLIARPNGNGNNWGVTIQHNGNWTWPTVTCTAN